European Patent Specification EP 3 724 329 B1, published August 20, 2025. Title: Peptidase and its uses. Applicant: Centre National de la Recherche Scientifique Commissariat à l'Energie Atomique et aux Energies Alternatives Université Grenoble Alpes. The sequence listing filed with the application follows.

SEQUENCE LISTING (16 sequences)

SEQ ID NO: 1 - protein, 350 aa, Methanococcus jannaschii
MSVVEYLKKLSKLHGISGREDSVREFMKKELEKYCDSVEIDNFGNLIAKRGNKGKKIMIAAHMDEIGLMVKYIDDNGFLKFTKIGGIYDPTILNQKVVVHGSKGDLIGVLGSKPPHRMKEEEKTKIIKYEDMFIDIGAESREEAIEMGVNIGTWVSFLSEVYDLGKNRLTGKAFDDRVGCAVLLEVMKRLSEEDIDCQVYAVGTVQEEVGLKGARVSAFKINPDVAIALDVTIAGDHPGIKKEDAPVDLGKGPVVGIVDASGRGLIAHPKVLDMIKAVSEKYKIDVQWEVGEGGTTDATAIHLTREGIPTGVISVPARYIHTPVEVIDKRDLEKTVELVYNCIKEVNNFF

SEQ ID NO: 2 - protein, 15 aa, Artificial Sequence
  synthetic peptide
YFLMNENRYTSWNSE

SEQ ID NO: 3 - protein, 6 aa, Artificial Sequence
  synthetic peptide
  MOD_RES (4)..(4): PHOSPHORYLATION
  NON_TER (6)..(6): linked to pNA
WFYSPR

SEQ ID NO: 4 - protein, 6 aa, Artificial Sequence
  synthetic peptide
MWAENK

SEQ ID NO: 5 - protein, 8 aa, Artificial Sequence
  artificial sequence
YDTSIVQR

SEQ ID NO: 6 - protein, 5 aa, Artificial Sequence
  artificial sequence
DAYPS

SEQ ID NO: 7 - protein, 75 aa, Artificial sequence
  partial dodecameric aminopeptidase
KIGGIYDPTILNQKVVVHGSKGDLIGVLGSKPPHRMKEEEKTKIIKYEDMFIDIGAESREEAIEMGVNIGTWVSF

SEQ ID NO: 8 - protein, 73 aa, Artificial sequence
  partial dodecameric aminopeptidase
KVGGIDDRLLYGRHVNVTTEKGILDGVIGATPPHLSLERDKSVIPWYDLVIDIGAESKEEALELVKPLDFAVF

SEQ ID NO: 9 - protein, 76 aa, Artificial sequence
  partial dodecameric aminopeptidase
PIGGVDPKTLIAQRFKVWIDKGKFIYGVGASVPPHIQKPEDRKKAPDWDQIFIDIGAESKEEAEDMGVKIGTVITW

SEQ ID NO: 10 - protein, 76 aa, Artificial sequence
  partial dodecameric aminopeptidase
PIGGVLPETLVAQRIRFFTEKGERYGVVGVLPPHLRRGQEDKGSKIDWDQIVVDVGASSKEEAEEMGFRVGTVGEF

SEQ ID NO: 11 - protein, 76 aa, Artificial sequence
  partial dodecameric aminopeptidase
PIGGVLPETLIAQKIRFFTEKGERYGVVGVLPPHLRREAKDQGGKIDWDSIIVDVGASSREEAEEMGFRIGTIGEF

SEQ ID NO: 12 - protein, 76 aa, Artificial sequence
  partial dodecameric aminopeptidase
PIGGVLERTLLYQRVVVRTRDGRLYRGVIGLKPPHVIKPEEAQKVPELRELFIDVGASSKEEVEKMGIRVGDIAVF

SEQ ID NO: 13 - protein, 76 aa, Artificial sequence
  partial dodecameric aminopeptidase
EIGGWNPMVVSSQRFKLLTRDGHEIPVISGSVPPHLTRGKGGPIMPAIADIVFDGGFADKAEAESFGIRPGDTIVP

SEQ ID NO: 14 - protein, 104 aa, Artificial sequence
  partial dodecameric aminopeptidase
EVYGGALFAPWFDRDLSLAGRVTFRANGKLESRLVDFRKAIAVIPNLAIHLNRAANEGWPINAQNELPPIIAQLAPGEAADFRLLLDEQLLREHGITADVVLDY

SEQ ID NO: 15 - protein, 120 aa, Artificial sequence
  partial dodecameric aminopeptidase
ETYGGGIWSTWFDRDLTLAGRVIVKCPTSGRLEQQLVHVERPILRIPHLAIHLQRNINENFGPNTEMHLVPILATAIQEELEKGTPEPGPLNAVDERHHSVLMSLLCAHLGLSPKDIVEM

SEQ ID NO: 16 - protein, 120 aa, Artificial sequence
  partial dodecameric aminopeptidase
ETYGGGIWSTWFDRDLTLAGRVIVKCPTSGRLEQRLVHVDRPILRIPHLAIHLQRNVNENFGPNMEMHLVPILATSIQEELEKGTPEPGPLNATDERHHSVLTSLLCAHLGLSPEDILEM